European Patent Application EP 4 631 958 A1, published October 15, 2025. Title: Peptide for cartilage regeneration and uses thereof. Applicant: CAREGEN CO., LTD. The sequence listing filed with the application follows.

SEQUENCE LISTING (12 sequences)

SEQ ID NO: 1 - DNA, 23 bp, synthetic construct
  source 1..23: mol_type = other DNA
ctatctggacgaagcagctggca

SEQ ID NO: 2 - DNA, 22 bp, synthetic construct
  source 1..22: mol_type = other DNA
atgggtgcaatgtcaatgatgg

SEQ ID NO: 3 - DNA, 20 bp, synthetic construct
  source 1..20: mol_type = other DNA
aactcagggcaggaggatgt

SEQ ID NO: 4 - DNA, 20 bp, synthetic construct
  source 1..20: mol_type = other DNA
tgtccttttggtcgtcgttc

SEQ ID NO: 5 - DNA, 20 bp, synthetic construct
  source 1..20: mol_type = other DNA
ccagcccgaacttgtaaaga

SEQ ID NO: 6 - DNA, 20 bp, synthetic construct
  source 1..20: mol_type = other DNA
tggacgcacaaccatcatac

SEQ ID NO: 7 - DNA, 20 bp, synthetic construct
  source 1..20: mol_type = other DNA
gcaggctatgagcagtgtga

SEQ ID NO: 8 - DNA, 20 bp, synthetic construct
  source 1..20: mol_type = other DNA
gcatacctcggaagcagaag

SEQ ID NO: 9 - DNA, 20 bp, synthetic construct
  source 1..20: mol_type = other DNA
accacagtccatgccatcac

SEQ ID NO: 10 - DNA, 20 bp, synthetic construct
  source 1..20: mol_type = other DNA
tccaccaccctgttgctgta

SEQ ID NO: 11 - DNA, 20 bp, synthetic construct
  source 1..20: mol_type = other DNA
gcggaggaagtcggtgaaga

SEQ ID NO: 12 - DNA, 20 bp, synthetic construct
  source 1..20: mol_type = other DNA
ccctctcgcttcaggtcagc